European Patent Specification EP 4 060 032 B1, published July 26, 2023. Title: Novel spermidine synthase variant and a method for producing L-valine using the same. Applicant: CJ CheilJedang Corporation. The sequence listing filed with the application follows.

SEQUENCE LISTING (11 sequences)

SEQ ID NO: 1 - protein, 513 aa, Artificial Sequence
  Spermidine synthase variant
MSDLGPIWRWLLLVSVSICAASGLVYELALVSLSTSLNGGGIVETSLIVAGYVAALGLGALLVKPFLNWPAQTFLGVETLLGLIGGCSALVLYFTFATIGQSLWILVIATAAIGILVGAELPLLMTMIQQGRLADAKTTGSLVATLNAADYLGALLGGLAWPFVLLPWLGMMRGAAAAGMINLVAALFVGCVLLRHLLPRTHFFVSVVALLLVIAALATVLVKSDGIVATARAQLYRDPVIYSHQSDYQDIVVTERGKDRRLYLNGGLQYSTRDQHRYTESLVYPSLNPEAESVLIIGGGDGLAARELLRFPSMQITQVELDPEVIEVANTVLRSDNGGAMEDPRVSIIVDDAFTWLRSGGNNGETYDSIIIDLPDPNNDTMARLYSEEFYTLARARLNEQGRMVVQSSSAYTTPDVFWRVGATLKSAGCEQVIPYHVHVPTFGDWGFQLCGPADMELELREDTPPLTFLNDEVLVAAGVFGLDNQPRELEPSTLDHPRVVEDLRKGYRESGD

SEQ ID NO: 2 - DNA, 1542 bp, Artificial Sequence
  Spermidine synthase variant coding gene
atgtctgatttaggacccatctggcgctggctgttattagtttccgtctccatttgtgcggcatcggggctggtctatgagctagccctggtgtccctttccaccagcttgaacggtggcggaattgtagaaacctccctcatcgtcgcaggttatgtagctgcccttggacttggtgcactgctggtcaagccgtttctcaactggcctgcacaaaccttcctcggtgtggaaaccttgctgggactcatcggtggttgctccgcgctggtgctatatttcacctttgcgaccatcggccagtccttgtggattctggtgattgccaccgctgcaattggcatcctggtcggcgctgaacttccactgctgatgaccatgatccagcaaggccgcctcgccgacgccaaaaccacaggatctctggttgccaccttgaatgctgctgattaccttggcgcacttttaggtggcctggcctggccttttgtgttgctgccgtggcttggcatgatgcgcggtgccgcagcagccggaatgatcaacctcgttgcagcactattcgtgggatgtgtgctgctgcgacatttgcttccgcgcacccacttcttcgtatccgtggtggcgcttcttctcgtgatcgcagcgcttgccaccgtgttggtgaaatccgacgggatcgttgccaccgcccgcgcacagctctaccgcgaccccgtgatctattcacaccaatctgactaccaagacatcgtagtgacagaacgaggcaaagaccgacgcctctacctcaatggcggtttgcagtattccactcgtgaccagcatagatatacagaatcactggtgtatccaagccttaatccagaggcagaatcggtgttaatcatcggcggtggcgatggcctcgcagcacgggaactcctccgattcccatcaatgcagatcacccaagttgaattagacccagaagtcatcgaagtagccaacacagtgctgcgctctgacaatgggggagcgatggaagatccccgcgtctccatcatcgttgacgacgctttcacctggctgcgctccggcggaaataatggcgaaacttacgattccatcatcatcgatcttcccgacccaaacaacgacaccatggccaggctgtattcagaagagttctacaccttggcccgagcacgactgaacgaacaaggccgcatggtggtgcaatcctccagcgcctacaccactccagatgtgttctggcgagttggagcaaccttgaaatcggcgggctgtgaacaagtcatcccatatcacgtgcatgttcccacatttggcgactggggcttccaactgtgtggccctgccgacatggaattagagcttcgggaagacaccccgccactgactttccttaatgatgaagttctggtggctgctggggtgtttgggttggataatcagcctcgtgaattggaaccttccacgctggatcatccccgcgtggtggaggatctgcgcaagggatatcgcgaatcaggcgactag

SEQ ID NO: 3 - protein, 513 aa, Artificial Sequence
  Wild-type spermidine synthase
MSDLGPIWRWLLLVSVSICAASGLVYELALVSLSTSLNGGGIVETSLIVAGYVAALGLGALLVKPFLNWPAQTFLGVETLLGLIGGCSALVLYFTFATIGQSLWILVIATAAIGILVGAELPLLMTMIQQGRLADAKTTGSLVATLNAADYLGALLGGLAWPFVLLPWLGMMRGAAAAGMINLVAALFVGCVLLRHLLPRTHFFVSVVALLLAIAALATVLVKSDGIVATARAQLYRDPVIYSHQSDYQDIVVTERGKDRRLYLNGGLQYSTRDQHRYTESLVYPSLNPEAESVLIIGGGDGLAARELLRFPSMQITQVELDPEVIEVANTVLRSDNGGAMEDPRVSIIVDDAFTWLRSGGNNGETYDSIIIDLPDPNNDTMARLYSEEFYTLARARLNEQGRMVVQSSSAYTTPDVFWRVGATLKSAGCEQVIPYHVHVPTFGDWGFQLCGPADMELELREDTPPLTFLNDEVLVAAGVFGLDNQPRELEPSTLDHPRVVEDLRKGYRESGD

SEQ ID NO: 4 - DNA, 1542 bp, Artificial Sequence
  Wild-type spermidine synthase coding gene
atgtctgatttaggacccatctggcgctggctgttattagtttccgtctccatttgtgcggcatcggggctggtctatgagctagccctggtgtccctttccaccagcttgaacggtggcggaattgtagaaacctccctcatcgtcgcaggttatgtagctgcccttggacttggtgcactgctggtcaagccgtttctcaactggcctgcacaaaccttcctcggtgtggaaaccttgctgggactcatcggtggttgctccgcgctggtgctatatttcacctttgcgaccatcggccagtccttgtggattctggtgattgccaccgctgcaattggcatcctggtcggcgctgaacttccactgctgatgaccatgatccagcaaggccgcctcgccgacgccaaaaccacaggatctctggttgccaccttgaatgctgctgattaccttggcgcacttttaggtggcctggcctggccttttgtgttgctgccgtggcttggcatgatgcgcggtgccgcagcagccggaatgatcaacctcgttgcagcactattcgtgggatgtgtgctgctgcgacatttgcttccgcgcacccacttcttcgtatccgtggtggcgcttcttctcgcgatcgcagcgcttgccaccgtgttggtgaaatccgacgggatcgttgccaccgcccgcgcacagctctaccgcgaccccgtgatctattcacaccaatctgactaccaagacatcgtagtgacagaacgaggcaaagaccgacgcctctacctcaatggcggtttgcagtattccactcgtgaccagcatagatatacagaatcactggtgtatccaagccttaatccagaggcagaatcggtgttaatcatcggcggtggcgatggcctcgcagcacgggaactcctccgattcccatcaatgcagatcacccaagttgaattagacccagaagtcatcgaagtagccaacacagtgctgcgctctgacaatgggggagcgatggaagatccccgcgtctccatcatcgttgacgacgctttcacctggctgcgctccggcggaaataatggcgaaacttacgattccatcatcatcgatcttcccgacccaaacaacgacaccatggccaggctgtattcagaagagttctacaccttggcccgagcacgactgaacgaacaaggccgcatggtggtgcaatcctccagcgcctacaccactccagatgtgttctggcgagttggagcaaccttgaaatcggcgggctgtgaacaagtcatcccatatcacgtgcatgttcccacatttggcgactggggcttccaactgtgtggccctgccgacatggaattagagcttcgggaagacaccccgccactgactttccttaatgatgaagttctggtggctgctggggtgtttgggttggataatcagcctcgtgaattggaaccttccacgctggatcatccccgcgtggtggaggatctgcgcaagggatatcgcgaatcaggcgactag

SEQ ID NO: 5 - DNA, 36 bp, Artificial Sequence
  speE_1F
tcgagctcggtaccccctccctcatcgtcgcaggtt

SEQ ID NO: 6 - DNA, 44 bp, Artificial Sequence
  speE_2R
cacggtggcaagcgctgcgatcacgagaagaagcgccaccacgg

SEQ ID NO: 7 - DNA, 44 bp, Artificial Sequence
  speE_3F
ccgtggtggcgcttcttctcgtgatcgcagcgcttgccaccgtg

SEQ ID NO: 8 - DNA, 36 bp, Artificial Sequence
  speE_4R
ctctagaggatccccctggccatggtgtcgttgttt

SEQ ID NO: 9 - DNA, 21 bp, Artificial Sequence
  speE_5F
cctccctcatcgtcgcaggtt

SEQ ID NO: 10 - DNA, 21 bp, Artificial Sequence
  speE_6R
ctggccatggtgtcgttgttt

SEQ ID NO: 11 - DNA, 5803 bp, Artificial Sequence
  pDCM2
gttcgcttgctgtccataaaaccgcccagtctagctatcgccatgtaagcccactgcaagctacctgctttctctttgcgcttgcgttttcccttgtccagatagcccagtagctgacattcatccggggtcagcaccgtttctgcggactggctttctacgtgttccgcttcctttagcagcccttgcgccctgagtgcttgcggcagcgtgaagctagcttttatcgccattcgccattcaggctgcgcaactgttgggaagggcgatcggtgcgggcctcttcgctattacgccagctggcgaaagggggatgtgctgcaaggcgattaagttgggtaacgccagggttttcccagtcacgacgttgtaaaacgacggccagtgaattcgagctcggtacccggggatcctctagagtcgacctgcaggcatgcaagcttggcgtaatcatggtcatagctgtttcctgtgtgaaattgttatccgctcacaattccacacaacatacgagccggaagcataaagtgtaaagcctggggtgcctaatgagtgagctaactcacattaattgcgttgcgctcactgcccgctttccagtcgggaaacctgtcgtgccagctgcattaatgaatcggccaacgcgcggggagaggcggtttgcgtattgggcgctcttccgcttcctcgctcactgactcgctgcgctcggtcgttcggctgcggcgagcggtatcagctcactcaaaggcggtaatacggttatccacagaatcaggggataacgcaggaaagaacatgtgagcaaaaggccagcaaaaggccaggaaccgtaaaaaggccgcgttgctggcgtttttccataggctccgcccccctgacgagcatcacaaaaatcgacgctcaagtcagaggtggcgaaacccgacaggactataaagataccaggcgtttccccctggaagctccctcgtgcgctctcctgttccgaccctgccgcttaccggatacctgtccgcctttctcccttcgggaagcgtggcgctttctcaatgctcacgctgtaggtatctcagttcggtgtaggtcgttcgctccaagctgggctgtgtgcacgaaccccccgttcagcccgaccgctgcgccttatccggtaactatcgtcttgagtccaacccggtaagacacgacttatcgccactggcagcagccactggtaacaggattagcagagcgaggtatgtaggcggtgctacagagttcttgaagtggtggcctaactacggctacactagaaggacagtatttggtatctgcgctctgctgaagccagttaccttcggaaaaagagttggtagctcttgatccggcaaacaaaccaccgctggtagcggtggtttttttgtttgcaagcagcagattacgcgcagaaaaaaaggatctcaagaagatcctttgatcttttctacggggtctgacgctcagtggaacgaaaactcacgttaagggattttggtcatgagattatcaaaaaggatcttcacctagatccttttggggtgggcgaagaactccagcatgagatccccgcgctggaggatcatccagccctgatagaaacagaagccactggagcacctcaaaaacaccatcatacactaaatcagtaagttggcagcatcacccgacgcactttgcgccgaataaatacctgtgacggaagatcacttcgcagaataaataaatcctggtgtccctgttgataccgggaagccctgggccaacttttggcgaaaatgagacgttgatcggcacgtaagaggttccaactttcaccataatgaaataagatcactaccgggcgtattttttgagttatcgagattttcaggagctgatagaaacagaagccactggagcacctcaaaaacaccatcatacactaaatcagtaagttggcagcatcacccgacgcactttgcgccgaataaatacctgtgacggaagatcacttcgcagaataaataaatcctggtgtccctgttgataccgggaagccctgggccaacttttggcgaaaatgagacgttgatcggcacgtaagaggttccaactttcaccataatgaaataagatcactaccgggcgtattttttgagttatcgagattttcaggagctctttggcatcgtctctcgcctgtcccctcagttcagtaatttcctgcatttgcctgtttccagtcggtagatattccacaaaacagcagggaagcagcgcttttccgctgcataaccctgcttcggggtcattatagcgattttttcggtatatccatcctttttcgcacgatatacaggattttgccaaagggttcgtgtagactttccttggtgtatccaacggcgtcagccgggcaggataggtgaagtaggcccacccgcgagcgggtgttccttcttcactgtcccttattcgcacctggcggtgctcaacgggaatcctgctctgcgaggctggccggctaccgccggcgtaacagatgagggcaagcggatggctgatgaaaccaagccaaccaggaagggcagcccacctatcaaggtgtactgccttccagacgaacgaagagcgattgaggaaaaggcggcggcggccggcatgagcctgtcggcctacctgctggccgtcggccagggctacaaaatcacgggcgtcgtggactatgagcacgtccgcgagggcgtcccggaaaacgattccgaagcccaacctttcatagaaggcggcggtggaatcgaaatctcgtgatggcaggttgggcgtcgcttggtcggtcatttcgaaaaaggttaggaatacggttagccatttgcctgcttttatatagttcantatgggattcacctttatgttgataagaaataaaagaaaatgccaataggatatcggcattttcttttgcgtttttatttgttaactgttaattgtccttgttcaaggatgctgtctttgacaacagatgttttcttgcctttgatgttcagcaggaagctcggcgcaaacgttgattgtttgtctgcgtagaatcctctgtttgtcatatagcttgtaatcacgacattgtttcctttcgcttgaggtacagcgaagtgtgagtaagtaaaggttacatcgttaggcggatcaagatccatttttaacacaaggccagttttgttcagcggcttgtatgggccagttaaagaattagaaacataaccaagcatgtaaatatcgttagacgtaatgccgtcaatcgtcatttttgatccgcgggagtcagtgaacaggtaccatttgccgttcattttaaagacgttcgcgcgttcaatttcatctgttactgtgttagatgcaatcagcggtttcatcacttttttcagtgtgtaatcatcgtttagctcaatcataccgagagcgccgtttgctaactcagccgtgcgttttttatcgctttgcagaagtttttgactttcttgacggaagaatgatgtgcttttgccatagtatgctttgttaaataaagattcttcgccttggtagccatcttcagttccagtgtttgcttcaaatactaagtatttgtggcctttatcttctacgtagtgaggatctctcagcgtatggttgtcgcctgagctgtagttgccttcatcgatgaactgctgtacattttgatacgtttttccgtcaccgtcaaagattgatttataatcctctacaccgttgatgttcaaagagctgtctgatgctgatacgttaacttgtgcagttgtcagtgtttgtttgccgtaatgtttaccggagaaatcagtgtagaataaacggatttttccgtcagatgtaaatgtggctgaacctgaccattcttgtgtttggtcttttaggatagaatcatttgcatcgaatttgtcgctgtctttaaagacgcggccagcgtttttccagctgtcaatagaagtttcgccgactttttgatagaacatgtaaatcgatgtgtcatccgcatttttaggatctccggctaatgcaaagacgatgtggtagccgtgatagtttgcgacagtgccgtcagcgttttgtaatggccagctgtcccaaacgtccaggccttttgcagaagagatatttttaattgtggacgaatcaaattcagaaacttgatatttttcatttttttgctgttcagggatttgcagcatatcatggcgtgtaatatgggaaatgccgtatgtttccttatatggcttttggttcgtttctttcgcaaacgcttgagttgcgcctcctgccagcagtgcggtagtaaaggttaatactgttgcttgttttgcaaactttttgatgttcatcgttcatgtctccttttttatgtactgtgttagcggtctgcttcttccagccctcctgtttgaagatggcaagttagttacgcacaataaaaaaagacctaaaatatgtaaggggtgacgccaaagtatacactttgccctttacacattttaggtcttgcctgctttatcagtaacaaacccgcgcgatttacttttcgacctcattctattagactctcgtttggattgcaactggtctattttcctcttttgtttgatagaaaatcataaaaggatttgcagactacgggcctaaagaactaaaaaatctatctgtttcttttcattctctgtattttttatagtttctgttgcatgggcataaagttgcctttttaatcacaattcagaaaatatcataatatctcatttcactaaataatagtgaacggcaggtatatgtgatgggttaaaaaggatcaccccagagtcccgctcagaagaactcgtcaagaaggcgatagaaggcgatgcgctgcgaatcgggagcggcgataccgtaaagcacgaggaagcggtcagcccattcgccgccaagctcttcagcaatatcacgggtagccaacgctatgtcctgatagcggtccgccacacccagccggccacagtcgatgaatccagaaaagcggccattttccaccatgatattcggcaagcaggcatcgccatgggtcacgacgagatcctcgccgtcgggcatccgcgccttgagcctggcgaacagttcggctggcgcgagcccctgatgctcttcgtccagatcatcctgatcgacaagaccggcttccatccgagtacgtgctcgctcgatgcgatgtttcgcttggtggtcgaatgggcaggtagccggatcaagcgtatgcagccgccgcattgcatcagccatgatggatactttctcggcaggagcaaggtgagatgacaggagatcctgccccggcacttcgcccaatagcagccagtcccttcccgcttcagtgacaacgtcgagacagctgcgcaaggaacgcccgtcgtggccagccacgatagccgcgctgcctcgtcttggagttcattcagggcaccggacaggtcggtcttgacaaaaagaaccgggcgcccctgcgctgacagccggaacacggcggcatcagagcagccgattgtctgttgtgcccagtcatagccgaatagcctctccacccaagcggccggagaacctgcgtgcaatccatcttgttcaatcatgcgaaacgatcctcatcctgtctcttgatcagatcttgatcccctgcgccatcagatccttggcggcaagaaagccatccagtttactttgcagggcttcccaaccttaccagagggcgccccagctggcaattccg